European Patent Application EP 4 800 036 A1, published September 2, 2026. Title: 结合Trop2的抗体或Trop2抗原结合片段以及抗Trop2 CAR和应用. Applicant: 上海优卡迪生物医药科技有限公司. The sequence listing filed with the application follows.

SEQUENCE LISTING (35 sequences)

SEQ ID NO: 1 - protein, 118 aa, Homo sapiens
EVQLVQSGGGLVQPGGSLRLSCEDSGFTFSSYWMSWVRQAPGKGLEWVSSISSSSSYIYYADSVKGRFTISRDNAKNSLYLQMNSLRGEDTAVYYCAREQSSSGFDYWGQGTLVTVSS

SEQ ID NO: 2 - protein, 107 aa, Homo sapiens
DIQMTQSPSTLSASVGDRVTITCRASQSISSWLAWYQQKPGKAPKLLIYKASSLESGVPPRFSGSGSGAEFTLTISSLQPDDFATYYCQQYNSYPLTFGGGTKVEVK

SEQ ID NO: 3 - protein, 8 aa, Homo sapiens
GFTFSSYW

SEQ ID NO: 4 - protein, 8 aa, Homo sapiens
ISSSSSYI

SEQ ID NO: 5 - protein, 11 aa, Homo sapiens
AREQSSSGFDY

SEQ ID NO: 6 - protein, 6 aa, Homo sapiens
QSISSW

SEQ ID NO: 7 - protein, 9 aa, Homo sapiens
QQYNSYPLT

SEQ ID NO: 8 - protein, 5 aa, Homo sapiens
SYWMS

SEQ ID NO: 9 - protein, 17 aa, Homo sapiens
SISSSSSYIYYADSVKG

SEQ ID NO: 10 - protein, 9 aa, Homo sapiens
EQSSSGFDY

SEQ ID NO: 11 - protein, 11 aa, Homo Sapiens
RASQSISSWLA

SEQ ID NO: 12 - protein, 7 aa, Homo sapiens
KASSLES

SEQ ID NO: 13 - protein, 9 aa, Homo sapiens
QQYNSYPLT

SEQ ID NO: 14 - protein, 7 aa, Homo sapiens
GFTFSSY

SEQ ID NO: 15 - protein, 6 aa, Homo sapiens
SSSSSY

SEQ ID NO: 16 - protein, 118 aa, Homo sapiens
ASTKGPSVFPLAPSSKSTSGGTAALGCLVKDYFPEPVTVSWNSGALTSGVHTFPAVLQSSGLYSLSSVVTVPSSSLGTQTYICNVNHKPSNTKVDKKVEPKSCDKTHTCPPCPAPELL

SEQ ID NO: 17 - protein, 105 aa, Homo sapiens
GGPSVFLFPPKPKDTLMISRTPEVTCVVVDVSHEDPEVKFNWYVDGVEVHNAKTKPREEQYNSTYRVVSVLTVLHQDWLNGKEYKCKVSNKALPAPIEKTISKAK

SEQ ID NO: 18 - protein, 107 aa, Homo sapiens
GQPREPQVYTLPPSRDELTKNQVSLTCLVKGFYPSDIAVEWESNGQPENNYKTTPPVLDSDGSFFLYSKLTVDKSRWQQGNVFSCSVMHEALHNHYTQKSLSLSPGK

SEQ ID NO: 19 - protein, 107 aa, Homo sapiens [sequence omitted]

SEQ ID NO: 20 - DNA, 354 bp, synthetic construct
  source 1..354: mol_type = other DNA
gaggtgcagctggtgcagtctgggggaggcttggtccagcccggggggtccctgagactctcctgtgaagactctggattcaccttcagtagctattggatgagctgggtccgccaggctccagggaaggggctggagtgggtctcatccattagtagtagtagtagttacatatactacgcagactcagtgaagggccgattcaccatctccagagacaacgccaagaactcactgtatctacagatgaacagcctgagaggcgaggacacggctgtttattactgtgcgagggaacagtctagcagtggctttgactactggggccagggaaccctggtcaccgtctcctca

SEQ ID NO: 21 - DNA, 321 bp, synthetic construct
  source 1..321: mol_type = other DNA
gacatccagatgacccagtctccttccaccctgtctgcatctgtaggagacagagtcaccatcacgtgccgggccagtcagagtattagtagctggttggcctggtatcagcagaaaccagggaaagcccctaaactcctgatctataaggcgtctagtttagaaagtggggtcccaccaaggttcagcggcagtggatctggggcagaattcactctcaccatcagcagcctgcagcctgatgattttgcaacttattactgccaacagtataatagttatccgctcactttcggcggagggaccaaggtggaggtcaaa

SEQ ID NO: 22 - DNA, 8251 bp, synthetic construct
  source 1..8251: mol_type = other DNA
agtgggaattggctccggtgcccgtcagtgggcagagcgcacatcgcccacagtccccgagaagttggggggaggggtcggcaattgaaccggtgcctagagaaggtggcgcggggtaaactgggaaagtgatgtcgtgtactggctccgcctttttcccgagggtgggggagaaccgtatataagtgcagtagtcgccgtgaacgttctttttcgcaacgggtttgccgccagaacacaggtaagtgccgtgtgtggttcccgcgggcctggcctctttacgggttatggcccttgcgtgccttgaattacttccacctggctgcagtacgtgattcttgatcccgagcttcgggttggaagtgggtgggagagttcgaggccttgcgcttaaggagccccttcgcctcgtgcttgagttgaggcctggcctgggcgctggggccgccgcgtgcgaatctggtggcaccttcgcgcctgtctcgctgctttcgataagtctctagccatttaaaatttttgatgacctgctgcgacgctttttttctggcaagatagtcttgtaaatgcgggccaagatctgcacactggtatttcggtttttggggccgcgggcggcgacggggcccgtgcgtcccagcgcacatgttcggcgaggcggggcctgcgagcgcggccaccgagaatcggacgggggtagtctcaagctggccggcctgctctggtgcctggcctcgcgccgccgtgtatcgccccgccctgggcggcaaggctggcccggtcggcaccagttgcgtgagcggaaagatggccgcttcccggccctgctgcagggagctcaaaatggaggacgcggcgctcgggagagcgggcgggtgagtcacccacacaaaggaaaagggcctttccgtcctcagccgtcgcttcatgtgactccacggagtaccgggcgccgtccaggcacctcgattagttctcgagcttttggagtacgtcgtctttaggttggggggaggggttttatgcgatggagtttccccacactgagtgggtggagactgaagttaggccagcttggcacttgatgtaattctccttggaatttgccctttttgagtttggatcttggttcattctcaagcctcagacagtggttcaaagtttttttcttccatttcaggtgtcgtgaggaagatctctagaagctgggtaccttgtgcccgggcgccaccatggagtttgggctgagctggctttttcttgtcgcgattcttaagggtgtccagtgcgagacgactcctcgacgaggaagcttgacatccagatgacccagagcccttccagcctgagcgctagcgtgggagacagggtgaccatcacctgcagggctagccaggatgtgagcaccgccgtggcctggtatcagcagaagcctggcaaggcccccaagctgctgatctacagcgccagcttcctgtacagcggagtgcccagcagattcagcggcagcggaagcggcaccgatttcaccctgaccatcagcagcctgcagcccgaggacttcgctacctactactgccagcagtacctgtaccaccccgccacctttggccagggcaccaaggtggagatcaagcgtacggtggctgcaccatctgtcttcatcttcccgccatctgatgagcagttgaaatctggaactgcctctgttgtgtgcctgctgaataacttctatcccagagaggccaaagtacagtggaaggtggataacgccctccaatcgggtaactcccaggagagtgtcacagagcaggacagcaaggacagcacctacagcctcagcagcaccctgacgctgagcaaagcagactacgagaaacacaaagtctacgcctgcgaagtcacccatcagggcctgagctcgcccgtcacaaagagcttcaacaggggagagtgtatccaaacggaggagcgtctccgcttcgaccaagggcccatcggtcttccccctggcaccctcctccaagagcacctctgggggcacagcggccctgggctgcctggtcaaggactacttccccgaaccggtgacggtgtcgtggaactcaggcgccctgaccagcggcgtgcacaccttcccggctgtcctacagtcctcaggactctactccctcagcagcgtggtgaccgtgccctccagcagcttgggcacccagacctacatctgcaacgtgaatcacaagcccagcaacaccaaggtggacaagaaagttgagcccaaatcttgtgacaaaactcacacatgcccaccgtgcccagcacctgaactcctggggggaccgtcagtcttcctcttccccccaaaacccaaggacaccctcatgatctcccggacccctgaggtcacatgcgtggtggtggacgtgagccacgaagaccctgaggtcaagttcaactggtacgtggacggcgtggaggtgcataatgccaagacaaagccgcgggaggagcagtacaacagcacgtaccgtgtggtcagcgtcctcaccgtcctgcaccaggactggctgaatggcaaggagtacaagtgcaaggtctccaacaaagccctcccagcccccatcgagaaaaccatctccaaagccaaagggcagccccgagaaccacaggtgtacaccctgcccccatcccgggatgagctgaccaagaaccaggtcagcctgacctgcctggtcaaaggcttctatcccagcgacatcgccgtggagtgggagagcaatgggcagccggagaacaactacaagaccacgcctcccgtgctggactccgacggctccttcttcctctacagcaagctcaccgtggacaagagcaggtggcagcaggggaacgtcttctcatgctccgtgatgcatgaggctctgcacaaccactacacgcagaagagcctctccctgtctccgggtaaatgagcggccgctcgaggccggcaaggccggatccagacatgataagatacattgatgagtttggacaaaccacaactagaatgcagtgaaaaaaatgctttatttgtgaaatttgtgatgctattgctttatttgtaaccattataagctgcaataaacaagttaacaacaacaattgcattcattttatgtttcaggttcagggggaggtgtgggaggttttttaaagcaagtaaaacctctacaaatgtggtatggctgattatgatccggctgcctcgcgcgtttcggtgatgacggtgaaaacctctgacacatgcagctcccggatacggtcacagcttgtctgtaagcggatgccgggagcagacaagcccgtcagggcgcgtcagcgggtgttggcgggtgtcggggcgcagccatgaggtcgactctagaggatcgatccccgccccggacgaactaaacctgactacgacatctctgccccttcttcgcggggcagtgcatgtaatcccttcagttggttggtacaacttgccaactgggccctgttccacatgtgacacggggggggaccaaacacaaaggggttctctgactgtagttgacatccttataaatggatgtgcacatttgccaacactgagtggctttcatcctggagcagactttgcagtctgtggactgcaacacaacattgcctttatgtgtaactcttggctgaagctcttacaccaatgctgggggacatgtacctcccaggggcccaggaagactacgggaggctacaccaacgtcaatcagaggggcctgtgtagctaccgataagcggaccctcaagagggcattagcaatagtgtttataaggcccccttgttaaccctaaacgggtagcatatgcttcccgggtagtagtatatactatccagactaaccctaattcaatagcatatgttacccaacgggaagcatatgctatcgaattagggttagtaaaagggtcctaaggaacagcgatatctcccaccccatgagctgtcacggttttatttacatggggtcaggattccacgagggtagtgaaccattttagtcacaagggcagtggctgaagatcaaggagcgggcagtgaactctcctgaatcttcgcctgcttcttcattctccttcgtttagctaatagaataactgctgagttgtgaacagtaaggtgtatgtgaggtgctcgaaaacaaggtttcaggtgacgcccccagaataaaatttggacggggggttcagtggtggcattgtgctatgacaccaatataaccctcacaaaccccttgggcaataaatactagtgtaggaatgaaacattctgaatatctttaacaatagaaatccatggggtggggacaagccgtaaagactggatgtccatctcacacgaatttatggctatgggcaacacataatcctagtgcaatatgatactggggttattaagatgtgtcccaggcagggaccaagacaggtgaaccatgttgttacactctatttgtaacaaggggaaagagagtggacgccgacagcagcggactccactggttgtctctaacacccccgaaaattaaacggggctccacgccaatggggcccataaacaaagacaagtggccactcttttttttgaaattgtggagtgggggcacgcgtcagcccccacacgccgccctgcggttttggactgtaaaataagggtgtaataacttggctgattgtaaccccgctaaccactgcggtcaaaccacttgcccacaaaaccactaatggcaccccggggaatacctgcataagtaggtgggcgggccaagataggggcgcgattgctgcgatctggaggacaaattacacacacttgcgcctgagcgccaagcacagggttgttggtcctcatattcacgaggtcgctgagagcacggtgggctaatgttgccatgggtagcatatactacccaaatatctggatagcatatgctatcctaatctatatctgggtagcataggctatcctaatctatatctgggtagcatatgctatcctaatctatatctgggtagtatatgctatcctaatttatatctgggtagcataggctatcctaatctatatctgggtagcatatgctatcctaatctatatctgggtagtatatgctatcctaatctgtatccgggtagcatatgctatcctaatagagattagggtagtatatgctatcctaatttatatctgggtagcatatactacccaaatatctggatagcatatgctatcctaatctatatctgggtagcatatgctatcctaatctatatctgggtagcataggctatcctaatctatatctgggtagcatatgctatcctaatctatatctgggtagtatatgctatcctaatttatatctgggtagcataggctatcctaatctatatctgggtagcatatgctatcctaatctatatctgggtagtatatgctatcctaatctgtatccgggtagcatatgctatcctcatgcatatacagtcagcatatgatacccagtagtagagtgggagtgctatcctttgcatatgccgccacctcccaagggggcgtgaattttcgctgcttgtccttttcctgctgcttatcgatgataagctgtcaaacatgagaattcttgaagacgaaagggcctcgtgatacgcctatttttataggttaatgtcatgataataatggtttcttagacgtcaggtggcacttttcggggaaatgtgcgcggaacccctatttgtttatttttctaaatacattcaaatatgtatccgctcatgagacaataaccctgataaatgcttcaataatattgaaaaaggaagagtatgagtattcaacatttccgtgtcgcccttattcccttttttgcggcattttgccttcctgtttttgctcacccagaaacgctggtgaaagtaaaagatgctgaagatcagttgggtgcacgagtgggttacatcgaactggatctcaacagcggtaagatccttgagagttttcgccccgaagaacgttttccaatgatgagcacttttaaagttctgctatgtggcgcggtattatcccgtgttgacgccgggcaagagcaactcggtcgccgcatacactattctcagaatgacttggttgagtactcaccagtcacagaaaagcatcttacggatggcatgacagtaagagaattatgcagtgctgccataaccatgagtgataacactgcggccaacttacttctgacaacgatcggaggaccgaaggagctaaccgcttttttgcacaacatgggggatcatgtaactcgccttgatcgttgggaaccggagctgaatgaagccataccaaacgacgagcgtgacaccacgatgcctgcagcaatggcaacaacgttgcgcaaactattaactggcgaactacttactctagcttcccggcaacaattaatagactggatggaggcggataaagttgcaggaccacttctgcgctcggcccttccggctggctggtttattgctgataaatctggagccggtgagcgtgggtctcgcggtatcattgcagcactggggccagatggtaagccctcccgtatcgtagttatctacacgacggggagtcaggcaactatggatgaacgaaatagacagatcgctgagataggtgcctcactgattaagcattggtaactgtcagaccaagtttactcatatatactttagattgatttaaaacttcatttttaatttaaaaggatctaggtgaagatcctttttgataatctcatgaccaaaatcccttaacgtgagttttcgttccactgagcgtcagaccccgtagaaaagatcaaaggatcttcttgagatcctttttttctgcgcgtaatctgctgcttgcaaacaaaaaaaccaccgctaccagcggtggtttgtttgccggatcaagagctaccaactctttttccgaaggtaactggcttcagcagagcgcagataccaaatactgttcttctagtgtagccgtagttaggccaccacttcaagaactctgtagcaccgcctacatacctcgctctgctaatcctgttaccagtggctgctgccagtggcgataagtcgtgtcttaccgggttggactcaagacgatagttaccggataaggcgcagcggtcgggctgaacggggggttcgtgcacacagcccagcttggagcgaacgacctacaccgaactgagatacctacagcgtgagctatgagaaagcgccacgcttcccgaagggagaaaggcggacaggtatccggtaagcggcagggtcggaacaggagagcgcacgagggagcttccagggggaaacgcctggtatctttatagtcctgtcgggtttcgccacctctgacttgagcgtcgatttttgtgatgctcgtcaggggggcggagcctatggaaaaacgccagcaacgcggcctttttacggttcctggccttttgctggccttttgctcacatgaagctgtccctgatggtcgtcatctacctgcctggacagcatggcctgcaacgcgggcatcccgatgccgccggaagcgagaagaatcataatggggaaggccatccagcctcgcgtcgcgaacgccagcaagacgtagcccagcgcgtcggccccgagatgcgccgcgtgcggctgctggagatggcggacgcgatggatatgttctgccaagggttggtttgcgcattcacagttctccgcaagaattgattggctccaattcttggagtggtgaatccgttagcgaggtgccgccctgcttcatccccgtggcccgttgctcgcgtttgctggcggtgtcactggccccgtgggttagggacggggtcccccatggggaatggtttatggttcgtgggggttattattttgggcgttgcgtggggtcaggtccacgactggactgagcagacagacccatggtttttggatggcctgggcatggaccgcatgtactggcgcgacacgaacaccgggcgtctgtggctgccaaacacccccgacccccaaaaaccaccgcgcggatttctggcgtgccaagctagtcgaccaattctcatgtttgacagcttatcatcgcagatccgggcaacgttgttgccattgctgcaggcgcagaactggtaggtatggaagatct

SEQ ID NO: 23 - DNA, 7930 bp, synthetic construct
  source 1..7930: mol_type = other DNA
agtgggaattggctccggtgcccgtcagtgggcagagcgcacatcgcccacagtccccgagaagttggggggaggggtcggcaattgaaccggtgcctagagaaggtggcgcggggtaaactgggaaagtgatgtcgtgtactggctccgcctttttcccgagggtgggggagaaccgtatataagtgcagtagtcgccgtgaacgttctttttcgcaacgggtttgccgccagaacacaggtaagtgccgtgtgtggttcccgcgggcctggcctctttacgggttatggcccttgcgtgccttgaattacttccacctggctgcagtacgtgattcttgatcccgagcttcgggttggaagtgggtgggagagttcgaggccttgcgcttaaggagccccttcgcctcgtgcttgagttgaggcctggcctgggcgctggggccgccgcgtgcgaatctggtggcaccttcgcgcctgtctcgctgctttcgataagtctctagccatttaaaatttttgatgacctgctgcgacgctttttttctggcaagatagtcttgtaaatgcgggccaagatctgcacactggtatttcggtttttggggccgcgggcggcgacggggcccgtgcgtcccagcgcacatgttcggcgaggcggggcctgcgagcgcggccaccgagaatcggacgggggtagtctcaagctggccggcctgctctggtgcctggcctcgcgccgccgtgtatcgccccgccctgggcggcaaggctggcccggtcggcaccagttgcgtgagcggaaagatggccgcttcccggccctgctgcagggagctcaaaatggaggacgcggcgctcgggagagcgggcgggtgagtcacccacacaaaggaaaagggcctttccgtcctcagccgtcgcttcatgtgactccacggagtaccgggcgccgtccaggcacctcgattagttctcgagcttttggagtacgtcgtctttaggttggggggaggggttttatgcgatggagtttccccacactgagtgggtggagactgaagttaggccagcttggcacttgatgtaattctccttggaatttgccctttttgagtttggatcttggttcattctcaagcctcagacagtggttcaaagtttttttcttccatttcaggtgtcgtgaggaagatctctagaagctgggtaccttgtgcccgggcgccaccatggacatgcgcgtgcccgcccagctgctgggcctgctgctgctgtggttccccggctcgcgatgcgagacgactcctcgacgaggaagcttatgcctccaccaagggacccagcgtgtttcccctggccccctgttccagatccacctccgaaagcacagccgctctcggctgcctggtcaaggattacttccctgagcccgtgacagtctcctggaatagcggcgctctgacctccggcgtgcataccttccctgctgtgctgcaatcctccggactgtacagcctgagcagcgtggtcaccgtgccttcctccagcctgggaaccaaaacctacacatgcaacgtggaccacaagcccagcaacaccaaagtggacaagagggtggagtccaagtacggacccccttgtcctccctgccctgctcctgaagccgctggaggacctagcgtgttcctgtttccccccaagcccaaggacaccctcatgatctccaggacccccgaggtgacctgtgtcgtggtggacgtgagccaagaggaccccgaggtgcagttcaactggtacgtggatggcgtcgaggtccataacgccaagaccaagcctagggaggagcagttcaacagcacctacagagtggtgagcgtcctgaccgtgctccaccaagactggctgaacggcaaggaatacaagtgcaaggtctccaacaagggactcccttcctccatcgagaagaccatcagcaaggccaagggccagcccagagaaccccaagtctacacactgccccccagccaagaggaaatgaccaagaaccaggtgagcctgacctgcctggtgaaaggcttctaccccagcgacattgctgtcgaatgggagagcaacggccaacccgagaacaactacaagaccaccccccctgtgctcgacagcgacggctccttcttcctctacagcaggctgacagtggacaagtccaggtggcaagagggcaatgtcttcagctgtagcgtcatgcacgaggccctccacaaccactacacccagaagagcctgtccctctccctgggctgaccaaacggaggagcgtctcccgtacggtggctgcaccatctgtcttcatcttcccgccatctgatgagcagttgaaatctggaactgcctctgttgtgtgcctgctgaataacttctatcccagagaggccaaagtacagtggaaggtggataacgccctccaatcgggtaactcccaggagagtgtcacagagcaggacagcaaggacagcacctacagcctcagcagcaccctgacgctgagcaaagcagactacgagaaacacaaagtctacgcctgcgaagtcacccatcagggcctgagctcgcccgtcacaaagagcttcaacaggggagagtgttgagcggccgctcgaggccggcaaggccggatccagacatgataagatacattgatgagtttggacaaaccacaactagaatgcagtgaaaaaaatgctttatttgtgaaatttgtgatgctattgctttatttgtaaccattataagctgcaataaacaagttaacaacaacaattgcattcattttatgtttcaggttcagggggaggtgtgggaggttttttaaagcaagtaaaacctctacaaatgtggtatggctgattatgatccggctgcctcgcgcgtttcggtgatgacggtgaaaacctctgacacatgcagctcccggatacggtcacagcttgtctgtaagcggatgccgggagcagacaagcccgtcagggcgcgtcagcgggtgttggcgggtgtcggggcgcagccatgaggtcgactctagaggatcgatccccgccccggacgaactaaacctgactacgacatctctgccccttcttcgcggggcagtgcatgtaatcccttcagttggttggtacaacttgccaactgggccctgttccacatgtgacacggggggggaccaaacacaaaggggttctctgactgtagttgacatccttataaatggatgtgcacatttgccaacactgagtggctttcatcctggagcagactttgcagtctgtggactgcaacacaacattgcctttatgtgtaactcttggctgaagctcttacaccaatgctgggggacatgtacctcccaggggcccaggaagactacgggaggctacaccaacgtcaatcagaggggcctgtgtagctaccgataagcggaccctcaagagggcattagcaatagtgtttataaggcccccttgttaaccctaaacgggtagcatatgcttcccgggtagtagtatatactatccagactaaccctaattcaatagcatatgttacccaacgggaagcatatgctatcgaattagggttagtaaaagggtcctaaggaacagcgatatctcccaccccatgagctgtcacggttttatttacatggggtcaggattccacgagggtagtgaaccattttagtcacaagggcagtggctgaagatcaaggagcgggcagtgaactctcctgaatcttcgcctgcttcttcattctccttcgtttagctaatagaataactgctgagttgtgaacagtaaggtgtatgtgaggtgctcgaaaacaaggtttcaggtgacgcccccagaataaaatttggacggggggttcagtggtggcattgtgctatgacaccaatataaccctcacaaaccccttgggcaataaatactagtgtaggaatgaaacattctgaatatctttaacaatagaaatccatggggtggggacaagccgtaaagactggatgtccatctcacacgaatttatggctatgggcaacacataatcctagtgcaatatgatactggggttattaagatgtgtcccaggcagggaccaagacaggtgaaccatgttgttacactctatttgtaacaaggggaaagagagtggacgccgacagcagcggactccactggttgtctctaacacccccgaaaattaaacggggctccacgccaatggggcccataaacaaagacaagtggccactcttttttttgaaattgtggagtgggggcacgcgtcagcccccacacgccgccctgcggttttggactgtaaaataagggtgtaataacttggctgattgtaaccccgctaaccactgcggtcaaaccacttgcccacaaaaccactaatggcaccccggggaatacctgcataagtaggtgggcgggccaagataggggcgcgattgctgcgatctggaggacaaattacacacacttgcgcctgagcgccaagcacagggttgttggtcctcatattcacgaggtcgctgagagcacggtgggctaatgttgccatgggtagcatatactacccaaatatctggatagcatatgctatcctaatctatatctgggtagcataggctatcctaatctatatctgggtagcatatgctatcctaatctatatctgggtagtatatgctatcctaatttatatctgggtagcataggctatcctaatctatatctgggtagcatatgctatcctaatctatatctgggtagtatatgctatcctaatctgtatccgggtagcatatgctatcctaatagagattagggtagtatatgctatcctaatttatatctgggtagcatatactacccaaatatctggatagcatatgctatcctaatctatatctgggtagcatatgctatcctaatctatatctgggtagcataggctatcctaatctatatctgggtagcatatgctatcctaatctatatctgggtagtatatgctatcctaatttatatctgggtagcataggctatcctaatctatatctgggtagcatatgctatcctaatctatatctgggtagtatatgctatcctaatctgtatccgggtagcatatgctatcctcatgcatatacagtcagcatatgatacccagtagtagagtgggagtgctatcctttgcatatgccgccacctcccaagggggcgtgaattttcgctgcttgtccttttcctgctgcttatcgatgataagctgtcaaacatgagaattcttgaagacgaaagggcctcgtgatacgcctatttttataggttaatgtcatgataataatggtttcttagacgtcaggtggcacttttcggggaaatgtgcgcggaacccctatttgtttatttttctaaatacattcaaatatgtatccgctcatgagacaataaccctgataaatgcttcaataatattgaaaaaggaagagtatgagtattcaacatttccgtgtcgcccttattcccttttttgcggcattttgccttcctgtttttgctcacccagaaacgctggtgaaagtaaaagatgctgaagatcagttgggtgcacgagtgggttacatcgaactggatctcaacagcggtaagatccttgagagttttcgccccgaagaacgttttccaatgatgagcacttttaaagttctgctatgtggcgcggtattatcccgtgttgacgccgggcaagagcaactcggtcgccgcatacactattctcagaatgacttggttgagtactcaccagtcacagaaaagcatcttacggatggcatgacagtaagagaattatgcagtgctgccataaccatgagtgataacactgcggccaacttacttctgacaacgatcggaggaccgaaggagctaaccgcttttttgcacaacatgggggatcatgtaactcgccttgatcgttgggaaccggagctgaatgaagccataccaaacgacgagcgtgacaccacgatgcctgcagcaatggcaacaacgttgcgcaaactattaactggcgaactacttactctagcttcccggcaacaattaatagactggatggaggcggataaagttgcaggaccacttctgcgctcggcccttccggctggctggtttattgctgataaatctggagccggtgagcgtgggtctcgcggtatcattgcagcactggggccagatggtaagccctcccgtatcgtagttatctacacgacggggagtcaggcaactatggatgaacgaaatagacagatcgctgagataggtgcctcactgattaagcattggtaactgtcagaccaagtttactcatatatactttagattgatttaaaacttcatttttaatttaaaaggatctaggtgaagatcctttttgataatctcatgaccaaaatcccttaacgtgagttttcgttccactgagcgtcagaccccgtagaaaagatcaaaggatcttcttgagatcctttttttctgcgcgtaatctgctgcttgcaaacaaaaaaaccaccgctaccagcggtggtttgtttgccggatcaagagctaccaactctttttccgaaggtaactggcttcagcagagcgcagataccaaatactgttcttctagtgtagccgtagttaggccaccacttcaagaactctgtagcaccgcctacatacctcgctctgctaatcctgttaccagtggctgctgccagtggcgataagtcgtgtcttaccgggttggactcaagacgatagttaccggataaggcgcagcggtcgggctgaacggggggttcgtgcacacagcccagcttggagcgaacgacctacaccgaactgagatacctacagcgtgagctatgagaaagcgccacgcttcccgaagggagaaaggcggacaggtatccggtaagcggcagggtcggaacaggagagcgcacgagggagcttccagggggaaacgcctggtatctttatagtcctgtcgggtttcgccacctctgacttgagcgtcgatttttgtgatgctcgtcaggggggcggagcctatggaaaaacgccagcaacgcggcctttttacggttcctggccttttgctggccttttgctcacatgaagctgtccctgatggtcgtcatctacctgcctggacagcatggcctgcaacgcgggcatcccgatgccgccggaagcgagaagaatcataatggggaaggccatccagcctcgcgtcgcgaacgccagcaagacgtagcccagcgcgtcggccccgagatgcgccgcgtgcggctgctggagatggcggacgcgatggatatgttctgccaagggttggtttgcgcattcacagttctccgcaagaattgattggctccaattcttggagtggtgaatccgttagcgaggtgccgccctgcttcatccccgtggcccgttgctcgcgtttgctggcggtgtcactggccccgtgggttagggacggggtcccccatggggaatggtttatggttcgtgggggttattattttgggcgttgcgtggggtcaggtccacgactggactgagcagacagacccatggtttttggatggcctgggcatggaccgcatgtactggcgcgacacgaacaccgggcgtctgtggctgccaaacacccccgacccccaaaaaccaccgcgcggatttctggcgtgccaagctagtcgaccaattctcatgtttgacagcttatcatcgcagatccgggcaacgttgttgccattgctgcaggcgcagaactggtaggtatggaagatct

SEQ ID NO: 24 - protein, 21 aa, synthetic construct
MALPVTALLLPLALLLHAARP

SEQ ID NO: 25 - protein, 240 aa, Homo sapiens
DIQMTQSPSTLSASVGDRVTITCRASQSISSWLAWYQQKPGKAPKLLIYKASSLESGVPPRFSGSGSGAEFTLTISSLQPDDFATYYCQQYNSYPLTFGGGTKVEVKGGGGSGGGGSGGGGSEVQLVQSGGGLVQPGGSLRLSCEDSGFTFSSYWMSWVRQAPGKGLEWVSSISSSSSYIYYADSVKGRFTISRDNAKNSLYLQMNSLRGEDTAVYYCAREQSSSGFDYWGQGTLVTVSS

SEQ ID NO: 26 - protein, 47 aa, synthetic construct
TTTPAPRPPTPAPTIASQPLSLRPEACRPAAGGAVHTRGLDFACDIY

SEQ ID NO: 27 - protein, 22 aa, synthetic construct
IWAPLAGTCGVLLLSLVITLYC

SEQ ID NO: 28 - protein, 42 aa, synthetic construct
KRGRKKLLYIFKQPFMRPVQTTQEEDGCSCRFPEEEEGGCEL

SEQ ID NO: 29 - protein, 112 aa, synthetic construct
RVKFSRSADAPAYKQGQNQLYNELNLGRREEYDVLDKRRGRDPEMGGKPRRKNPQEGLYNELQKDKMAEAYSEIGMKGERRRGKGHDGLYQGLSTATKDTYDALHMQALPPR

SEQ ID NO: 30 - DNA, 63 bp, synthetic construct
  source 1..63: mol_type = other DNA
atggccttaccagtgaccgccttgctcctgccgctggccttgctgctccacgccgccaggccg

SEQ ID NO: 31 - DNA, 720 bp, synthetic construct
  source 1..720: mol_type = other DNA
gacatccagatgacccagtctccttccaccctgtctgcatctgtaggagacagagtcaccatcacgtgccgggccagtcagagtattagtagctggttggcctggtatcagcagaaaccagggaaagcccctaaactcctgatctataaggcgtctagtttagaaagtggggtcccaccaaggttcagcggcagtggatctggggcagaattcactctcaccatcagcagcctgcagcctgatgattttgcaacttattactgccaacagtataatagttatccgctcactttcggcggagggaccaaggtggaggtcaaaggtggcggtggctcgggcggtggtgggtcgggtggcggcggatctgaggtgcagctggtgcagtctgggggaggcttggtccagcccggggggtccctgagactctcctgtgaagactctggattcaccttcagtagctattggatgagctgggtccgccaggctccagggaaggggctggagtgggtctcatccattagtagtagtagtagttacatatactacgcagactcagtgaagggccgattcaccatctccagagacaacgccaagaactcactgtatctacagatgaacagcctgagaggcgaggacacggctgtttattactgtgcgagggaacagtctagcagtggctttgactactggggccagggaaccctggtcaccgtctcctca

SEQ ID NO: 32 - DNA, 141 bp, synthetic construct
  source 1..141: mol_type = other DNA
accacgacgccagcgccgcgaccaccaacaccggcgcccaccatcgcgtcgcagcccctgtccctgcgcccagaggcgtgccggccagcggcggggggcgcagtgcacacgagggggctggacttcgcctgtgatatctac

SEQ ID NO: 33 - DNA, 66 bp, synthetic construct
  source 1..66: mol_type = other DNA
atctgggcgcccttggccgggacttgtggggtccttctcctgtcactggttatcaccctttactgc

SEQ ID NO: 34 - DNA, 126 bp, synthetic construct
  source 1..126: mol_type = other DNA
aaacggggcagaaagaaactcctgtatatattcaaacaaccatttatgagaccagtacaaactactcaagaggaagatggctgtagctgccgatttccagaagaagaagaaggaggatgtgaactg

SEQ ID NO: 35 - DNA, 336 bp, synthetic construct
  source 1..336: mol_type = other DNA
agagtgaagttcagcaggagcgcagacgcccccgcgtacaagcagggccagaaccagctctataacgagctcaatctaggacgaagagaggagtacgatgttttggacaagagacgtggccgggaccctgagatggggggaaagccgagaaggaagaaccctcaggaaggcctgtacaatgaactgcagaaagataagatggcggaggcctacagtgagattgggatgaaaggcgagcgccggaggggcaaggggcacgatggcctttaccagggtctcagtacagccaccaaggacacctacgacgcccttcacatgcaggccctgccccctcgc